European Patent Specification EP 3 921 336 B1, published March 1, 2023. Title: GLUCAGON ANALOG AGONISTS AND METHODS OF USING THE SAME. Applicant: Eli Lilly and Company. The sequence listing filed with the application follows.

SEQUENCE LISTING (9 sequences)

SEQ ID NO: 1 - protein, 29 aa, Homo sapiens
HSQGTFTSDYSKYLDSRRAQDFVQWLMNT

SEQ ID NO: 2 - protein, 29 aa, Artificial Sequence
  Synthetic Construct
  VARIANT (3)..(3): Xaa at position 3 is Q or Dab(Ac)
  MISC_FEATURE (16)..(16): Xaa at position 16 is Aib
  VARIANT (21)..(21): Xaa at position 21 is Q or A
  MISC_FEATURE (25)..(25): Xaa at position 25 is 4-Pal
HSXGTFTSDYSKYLDXRRAQXFVKXLLST

SEQ ID NO: 3 - protein, 29 aa, Artificial Sequence
  Synthetic Construct
  MISC_FEATURE (16)..(16): Xaa at position 16 is Aib
  MISC_FEATURE (25)..(25): Xaa at position 25 is 4-Pal
HSQGTFTSDYSKYLDXRRAQQFVKXLLST

SEQ ID NO: 4 - protein, 29 aa, Artificial Sequence
  Synthetic Construct
  MISC_FEATURE (16)..(16): Xaa at position 16 is Aib
  MISC_FEATURE (25)..(25): Xaa at position 25 is 4-Pal
HSQGTFTSDYSKYLDXRRAQAFVKXLLST

SEQ ID NO: 5 - protein, 29 aa, Artificial Sequence
  Synthetic Construct
  MISC_FEATURE (3)..(3): Xaa at position 3 is Dab(Ac)
  MISC_FEATURE (16)..(16): Xaa at position 16 is Aib
  MISC_FEATURE (25)..(25): Xaa at position 25 is 4-Pal
HSXGTFTSDYSKYLDXRRAQAFVKXLLST

SEQ ID NO: 6 - protein, 29 aa, Artificial Sequence
  Synthetic Construct
  MISC_FEATURE (3)..(3): Xaa at position 3 is Dab(Ac)
  MISC_FEATURE (16)..(16): Xaa at position 16 is Aib
  MISC_FEATURE (25)..(25): Xaa at position 25 is 4-Pal
HSXGTFTSDYSKYLDXRRAQQFVKXLLST

SEQ ID NO: 7 - protein, 42 aa, Homo sapiens
  MOD_RES (42)..(42): AMIDATION
YAEGTFISDYSIAMDKIHQQDFVNWLLAQKGKKNDWKHNITQ

SEQ ID NO: 8 - protein, 30 aa, Homo sapiens
  MOD_RES (30)..(30): AMIDATION
HAEGTFTSDVSSYLEGQAAKEFIAWLVKGR

SEQ ID NO: 9 - protein, 34 aa, Homo sapiens
HADGSFSDEMNTILDNLAARDFINWLIQTKITDR